European Patent Application EP 4 269 401 A1, published November 1, 2023. Title: GLYCINE N-METHYLTRANSFERASE SPECIFIC ENHANCER, PREPARATION METHOD AND USE THEREOF. Applicant: Chen, Yi-Ming Tzeng, Cherng-Chyi Chen, Yeh-Long Tseng, Chih-Hua Yen, Chia-Hung Rajni Kant Yang, Ming-Hui. The sequence listing filed with the application follows.

SEQUENCE LISTING (11 sequences)

SEQ ID NO: 1 - DNA, 21 bp, Artificial sequence
  TBP forward primer
tgcacaggagccaagagtgaa

SEQ ID NO: 2 - DNA, 20 bp, Artificial sequence
  TBP reverse primer
cacatcacagctccccacca

SEQ ID NO: 3 - DNA, 22 bp, Artificial sequence
  MYC forward primer
ttcggttgttgctgatctgtct

SEQ ID NO: 4 - DNA, 21 bp, Artificial sequence
  MYC reverse primer
ccctccactcggaaggactat

SEQ ID NO: 5 - DNA, 18 bp, Artificial sequence
  p21 forward primer
tgagccgcgactgtgatg

SEQ ID NO: 6 - DNA, 23 bp, Artificial sequence
  p21 reverse primer
gtctcggtgacaaagtcgaagtt

SEQ ID NO: 7 - DNA, 25 bp, Artificial sequence
  p27 forward primer
tgcaaccgacgattcttctactcaa

SEQ ID NO: 8 - DNA, 29 bp, Artificial sequence
  p27 reverse primer
caagcagtgatgtatctgataaacaagga

SEQ ID NO: 9 - DNA, 19 bp, Artificial sequence
  GNMT forward primer
actggatgactctggacaa

SEQ ID NO: 10 - DNA, 17 bp, Artificial sequence
  GNMT reverse primer
actgaggatgtggtcgt

SEQ ID NO: 11 - RNA, 21 nt, Artificial sequence
  MYC-lentiviral shRNA
cctgagacagatcagcaacaa